European Patent Application EP 4 717 768 A1, published April 1, 2026. Title: 一种植物根肿菌响应启动子及其应用. Applicant: 中国科学院遗传与发育生物学研究所. The sequence listing filed with the application follows.

SEQUENCE LISTING (23 sequences)

SEQ ID NO: 1 - DNA, 447 bp, synthetic construct
  source 1..447: mol_type = other DNA
atggagactgtctccgccgttaaccaaacactccccatctccggcggtgaaccggtgaagttcacgacatactctgccgcagttcacaaagtccttgtcatggtcaacgccggaattctagggttactccagcttgtcagccaacagtcctctgttttggaaacacataaagccgcattcctttgtttctgtgttttcattctattctacgccgttcttcgcgtccgtgaagccatggacgtgcgcctacaacccggtttagtcccaaggctcattggacatgggagccatctcttcggtggtctagccgctcttgtgctcgtctccgtcgttagtaccgcgttttctattgtcctttttcttctctggtttatctggctctccgccgtcgtctacttagagacaaacaaacccagtgcctgtccacctcagttaccaccagtttaa

SEQ ID NO: 2 - DNA, 447 bp, synthetic construct
  source 1..447: mol_type = other DNA
atggagactgtctccgccgttaaccaaacactccccatctccggcggtgaaccggtgaagttcacgacatactctgccgcagttcacaaagtccttgtcatgatcaacgccggaattctagggttactccagcttgtcagccaacagtcctctgttttggaaacacataaagccgcattcctttgtttctgtgttttcattctattctacgccgttcttcgcgtccgtgaagccatggacgtgcgcctacaacccggtttagtcccaaggctcattggacatgggagccatctcttcggtggtctagccgctcttgtactcgtctccgtcgttagtaccgcattttctattgtcctttttcttctctggtttatctggctctccgccgtcgtctacttggagacaaacaaacccagtgcctgtccacctcagttaccaccagtttaa

SEQ ID NO: 3 - DNA, 3727 bp, synthetic construct
  source 1..3727: mol_type = other DNA
agccagacaaactcccatctcttagataaaacgcttgtcttaatcgaatctttgatcccaaggtatgagactatcttagctaatgatctggtaatgcgctgattctatcgcactccattatcgctacaaaaacaaggacaatatcaacaagaagaacgaaccatatgccttgagagtttctcaattaattccaaaaactagggtttattaaagtcggttaaaaaacaacatgagctagttctatagcactctatcgcttaaagataaagaaaaacaacgacaaaataaaccaacaaagtcgaatcatatgccttgagagtttgttgagtatacttacaatcgagggaggaggaatgaagaacgtaactaaccgacggtcaagtgaatatggccggagatctagctttaaggtgagcaagtgatacctactatatagtttatatagtttttcataaagacctttacaaggataacatttacaaaaacatttaccattataattaaatacattagctttttaatatatttcttaattttattaattatacatagatatgttttctattttattgagaacaaaatcttctcaaaatctagttgtcaaattttcattcaacttttaattataaaaaataagaaatttaaaagtaacttgtattcaaaaatgtcaaattaacaaaaaaattgtggtctcacacattattttctaactgctattcttaaattcgcaactaatatttgcttaatcaaatttactttcattttgaaataattatattttatccaaaaaaaggactattgtaaaataaatcaagattttttaaactaatattataatatatcaagatatttttatataattccattaaaaatctataatccccatcaaaattgattctatcatttgattattatttattaagattatatatcttattatataaatcttagttttcaaatatgtaaggaatataatttaacatatattaagtactcaataaaatttagttgcaaatatttatgtgtttatgatatcaacatattcaactaaacaattaataaggaggtaacatgtgttttaaaaattgtatgaaatgtgaaagtttgctcactcatattttgatcatccagttccagctaaactaaagaagttaaggtcccataaccgagaagtttgtcaaaagtttttattagatatttttaaatttaagaaacagataaactttacatggatttatcaatatcttcagatactttagataagtccattgaccacggcaaaggattattttaaagtacgtgaaaaaacattaagaaacagaaacaaaaagaaaaatgaaaagtttcgggaatgtttggatatcaagtaaataaaatgaattcgaagccttctctctttagaacttcgagtttttcgtctgataacgatgtttacgtattattatgatcatctcgcggctgcggagaaggacataagctcgaataatttctgtagtttggtggatgcttccgttatgttatacgacgaagaacaccgtgatcttcttccaaagaaagtaaactccagatgccaagcgaagacaaagaaacaagaaaaagagagtgacaagagattcttccatctcttccctaaaaaaagaagaacttcggttgttactgtaagaaccctgaacaaaaccaacaaaatctttataggatttctatttcttcatcgctcctcgaccttaacacgatccccggtgattcttctgacccacgtaacgaacttcaagggctttattattcttcttcttcatcgtttcttggagattacaagatcactgctgattacaagatgaaaaacccacaaacccctccttcttcttcaactttacttgttgagtacaacaccgagatgacaaaccctaattctcagacaaacagcaagagaaagtgtagtgctaatggtagtgaatccagtccagagccgtctcttaatgcctttcaacaccctaattcgtaacgactttttgacgcctgttgagtcgagaatcctactagaagaagatgacacggagggagttggagcgactctagtggatccatgggaggtaaagtggggtgtttttttgaagaaacggaagatgaagaaagattcagggaaaggaagcttgaattacgctattatctgcggatggaacgatatcgttgaggctaacgtattggaaaaagtcgatgacatcagtatttggtcttgatcaagtgtggatgatcaaggaagtaagatcttgatcaaggaagtaagatcttgatcaattcacagataatcggacggtcaccatttcacaggtatgcttcttagaattctcctataaacgagagttgaaagatcatgtttagcaactgatacaaaattgacatcaattataatatgggcaattgacaaaaataacaccaaaaaaattttcttccaatattaacacaatatttctaaaatttcacaaatagcactataaacttcaattaaacttaactaaaatataagatagaaaataaaaatgagagcagacactaatctaatattaaattgaatcaaataattttaaatagtggaaatatatactctaaattgaaaataaagaactcaaatataatactacaaactaatatttaaataaaaaatctcttttaaatggtgaaaatatataccctaaattagaaataggaaacccaaatataaaaccataaactaatattaaaatgaatcaaaattttcttaaatgattgaaatatataccctaaattggatatagagaaaccaaatataatattttaaatttatttctaatttattttggttgaatagattttatataaaaattatggtattattgagaaataaattagtgataatatttttagaataaaagctttatagtaagccaagtagtgctatttttgaaagtttatgaagtgtgcgttattattgttcataaaatttattttagtgctatttttaagaatttctcttataataatcgatttaagtattttgattattaacatcagtcagtaataatcttatgcaaattatatgcatcaccaatatataaatcacttatttaagtgatgcaaaatttttttacattatttttttaactaatgcaaatatttataataaatgatgtaaaacaatttttttttttagtgaaagtgaaagtgaattgaaagtgaagactagaaaaatcttgatcgttgcacaagccgagccgatgacagtcccttacacatgtgtttttggagccgatgactgtcatttttagataagtgtggaaagtggcttctatgtttttggagccgatgactgtcatttttagataagtgtggaaagtggcttctattcaaggaaggaaagtcaagccgagtatgatcttgatcaattcacagataatcggacggtcaccatttcacaggtatgcttcttagatttcttcttagatgtcacaggtgacgatgacagtcccttacacatgtgtttttggagctcctcacaggtgacgatgacagtcccttacacaggtgacgatgacagtccctttctttttatttatctttttttttattattgtaagggcctcttagatttctcctataaaacgagagttagaaagatcaagaaaatggtgcacaaaaaaaaaaacgaaagatcaagaaaacaaaagagaataaaactgcaaagatacaaatt

SEQ ID NO: 4 - DNA, 3036 bp, synthetic construct
  source 1..3036: mol_type = other DNA
agccacacaaactcccatctcttagataaaacgcttgtcttaatcgaatctttgatcccaaggtatgagactatcttagctaccaaatgatctggtaatgcgctgattctatcgcactccatgatcactacaaaaaacaaggacaatatcaacaagaagaacgaaccctatgccttgagagtttctcaattaattccaaaaactagggtttattaaagtcggttaaaaaacaacatgagctagttctatagcactctatcgcttaaagataaagaaaaacaacgacaaaataaaccaacaaagtcgaatcatatgccttgagagtttgttgagtaaacttacaatcgagggaggaggaatgaagaacgtaactaaccgacggtcaagtgaatatggccagagatctagctttaaggtgagcaagtgatacctactatatagtttatatagtttttcataaagacctttacaaggataacacttacaaaaacatttaccattataattaaatacattagctttttaatatatttcttaattttattaattataaatagatatgttgtcaacttttcattcaactttttattattaaaaaaaagaaatttaaaagtgacttgtattcaaaaatgtcaaattaacaaaaaaaagtgtggtttcacacattattttagaaactgctattcataaattcacacatatttgcttgataaaatttactttcattttaaattaattatattttatccaaaaaaggactattgtaaaataaatcaagatttctaaactaatatgataatatatcaagatatttttatataattccattaaaaatctataatcaccattaaaattgattctatcatttgattattttttagtaagattatatatcttattatataaatcttagttttcaatatgtaaggaatataatttaacatacattaagtactcaataaaatttagttgcaaatatttatgtgtttatgatatcaacatattcaactaaacaattaataaggaggtaacatgtgttttaaaaattgtatgaaatgtgaaagtttgctcactcatattttgatcttccagttccagctaaactaaagaagttaaggtcccataaccgagaagtttgtcaaaagtttatattagatatttttaaatttaagaaacagataaactttacatggatttatcaatatcttcagatactttagataagtccattgaccacggtaaaggattattttaaagtacgtgaaaaaacattaagaaacagaaacaaaaagaaaaatgaaaagtttcgggaatgcttgggtatcaagtaaataaaatgaattcgaagccttctctctttagaacttcgagtttttggtctgataacgatgtttacgtattattatgatcatctcgcggctgcgtagaaggacataagctcgaataatttctgtagtttggtggatgcttccgatatgttatacgacgaagaacaccgtgatcttcttccaaagaaagtaaactccagatgccaagcgaagacaaagaaacaagaaaaagagagtgacaagagattcttccatctcttccctaaaaaaagaagaacttcggttgttactgtaagaaccctgaacaaaaccaacaaaatctttataggatttctacttcttcatcgctcctcgaccttaacacgatccccggtgattcttctgacccacgtaacgaacttcaagggctttattcttcttcttcttcatcgtttcttggagattacaagatcactgctgattacaagatgaaaaacccacaaacccctccttcttcttcaactttacttgttgagtacaacaccgagatgacaaacccaccaaaccctaattctcatacaaacagcaagagaaagtgtagtgctaatggtagtgaatccagtccagagccgtctcttaatgcctttcaacaccctaattcgtaacgactttttgacgcctgttgagtcgagaatcctactagaagaagatgacacggagggagttggagcgactctagtggatccatgtgaggtaaagtggggtgtttttttgaagaaacggaagatgaagaaagattcagggaaagaaagcttgaattacgctattatctgcgggtggaacgatatcgttgaggctaacgtattggaaaaagacgatgacatcagtatttggtctttcaggcggggtataaatggaatcctttcctttgcccttgttcttcctcctcctcctgacatgccatagagtatctcttcccatgctctttgtctctcacaagtttcttgattgatttattcgcactgtgagttttaattttggtctagtttttctttttctcttttttttttataagtctaaatccggaaataacccaatacccaatatccggaaataaataaatttatttataaaattgaatatcttttaacaacaaaaaaaaagaacaaaaaggatcatttgtcctttcattacaaaatgagcattactattcattctataatgaaatgatatttttttgtgttttatccaatatagaagtttgttagcagatgacaaaaaaaaaaaaaaaagtttgtcgcgaaaatataatcaaagtctggtgctgagtcaaatatgaattgaaagtgaagactagaaaaatcttcatcggacggtcatttttagataagtggggaaagtggcttctatgcaaggaaggaaagggaagtcgccgacaggcaaacgaacaggcccaattcatagataatcggacggtcgccatcacatgtttacgaaagcaataacaaaaacaaaacaaaaacaatattttaaccaagtatgtgtgttttaattttttaacatttgaccatgtgttttttagtttacatacgtgtttttggagcccttctctcccctgtctcttagatttctcctataaaacacccaaggaaagatcaagaaaatggtgcacaaaaaaaaaagaaagatcaagaaaacaaaagagaataaaactgcgaagatacaaatt

SEQ ID NO: 5 - DNA, 5147 bp, synthetic construct
  source 1..5147: mol_type = other DNA
agccagacaaactcccatctcttagataaaacgcttgtcttaatcgaatctttgatcccaaggtatgagactatcttagctaatgatctggtaatgcgctgattctatcgcactccattatcgctacaaaaacaaggacaatatcaacaagaagaacgaaccatatgccttgagagtttctcaattaattccaaaaactagggtttattaaagtcggttaaaaaacaacatgagctagttctatagcactctatcgcttaaagataaagaaaaacaacgacaaaataaaccaacaaagtcgaatcatatgccttgagagtttgttgagtatacttacaatcgagggaggaggaatgaagaacgtaactaaccgacggtcaagtgaatatggccggagatctagctttaaggtgagcaagtgatacctactatatagtttatatagtttttcataaagacctttacaaggataacatttacaaaaacatttaccattataattaaatacattagctttttaatatatttcttaattttattaattatacatagatatgttttctattttattgagaacaaaatcttctcaaaatctagttgtcaaattttcattcaacttttaattataaaaaataagaaatttaaaagtaacttgtattcaaaaatgtcaaattaacaaaaaaattgtggtctcacacattattttctaactgctattcttaaattcgcaactaatatttgcttaatcaaatttactttcattttgaaataattatattttatccaaaaaaaggactattgtaaaataaatcaagattttttaaactaatattataatatatcaagatatttttatataattccattaaaaatctataatccccatcaaaattgattctatcatttgattattatttattaagattatatatcttattatataaatcttagttttcaaatatgtaaggaatataatttaacatatattaagtactcaataaaatttagttgcaaatatttatgtgtttatgatatcaacatattcaactaaacaattaataaggaggtaacatgtgttttaaaaattgtatgaaatgtgaaagtttgctcactcatattttgatcatccagttccagctaaactaaagaagttaaggtcccataaccgagaagtttgtcaaaagtttttattagatatttttaaatttaagaaacagataaactttacatggatttatcaatatcttcagatactttagataagtccattgaccacggcaaaggattattttaaagtacgtgaaaaaacattaagaaacagaaacaaaaagaaaaatgaaaagtttcgggaatgtttggatatcaagtaaataaaatgaattcgaagccttctctctttagaacttcgagtttttcgtctgataacgatgtttacgtattattatgatcatctcgcggctgcggagaaggacataagctcgaataatttctgtagtttggtggatgcttccgttatgttatacgacgaagaacaccgtgatcttcttccaaagaaagtaaactccagatgccaagcgaagacaaagaaacaagaaaaagagagtgacaagagattcttccatctcttccctaaaaaaagaagaacttcggttgttactgtaagaaccctgaacaaaaccaacaaaatctttataggatttctatttcttcatcgctcctcgaccttaacacgatccccggtgattcttctgacccacgtaacgaacttcaagggctttattattcttcttcttcatcgtttcttggagattacaagatcactgctgattacaagatgaaaaacccacaaacccctccttcttcttcaactttacttgttgagtacaacaccgagatgacaaaccctaattctcagacaaacagcaagagaaagtgtagtgctaatggtagtgaatccagtccagagccgtctcttaatgcctttcaacaccctaattcgtaacgactttttgacgcctgttgagtcgagaatcctactagaagaagatgacacggagggagttggagcgactctagtggatccatgggaggtaaagtggggtgtttttttgaagaaacggaagatgaagaaagattcagggaaaggaagcttgaattacgctattatctgcggatggaacgatatcgttgaggctaacgtattggaaaaagtcgatgacatcagtatttggtcttgatcaagtgtggatgatcaaggaagtaagatcttgatcaaggaagtaagatcttgatcaattcacagataatcggacggtcaccatttcacaggtatgcttcttagaattctcctataaacgagagttgaaagatcatgtttagcaactgatacaaaattgacatcaattataatatgggcaattgacaaaaataacaccaaaaaaattttcttccaatattaacacaatatttctaaaatttcacaaatagcactataaacttcaattaaacttaactaaaatataagatagaaaataaaaatgagagcagacactaatctaatattaaattgaatcaaataattttaaatagtggaaatatatactctaaattgaaaataaagaactcaaatataatactacaaactaatatttaaataaaaaatctcttttaaatggtgaaaatatataccctaaattagaaataggaaacccaaatataaaaccataaactaatattaaaatgaatcaaaattttcttaaatgattgaaatatataccctaaattggatatagagaaaccaaatataatattttaaatttatttctaatttattttggttgaatagattttatataaaaattatggtattattgagaaataaattagtgataatatttttagaataaaagctttatagtaagccaagtagtgctatttttgaaagtttatgaagtgtgcgttattattgttcataaaatttattttagtgctatttttaagaatttctcttataataatcgatttaagtattttgattattaacatcagtcagtaataatcttatgcaaattatatgcatcaccaatatataaatcacttatttaagtgatgcaaaatttttttacattatttttttaactaatgcaaatatttataataaatgatgtaaaacaatttttttttttagtgaaagtgaaagtgaattgaaagtgaagactagaaaaatcttgatcgttgcacaagccgagccgatgacagtcccttacacatgtgtttttggagccgatgactgtcatttttagataagtgtggaaagtggcttctatgtttttggagccgatgactgtcatttttagataagtgtggaaagtggcttctattcaaggaaggaaagtcaagccgagtatgatcttgatcaattcacagataatcggacggtcaccatttcacaggtatgcttcttagatttcttcttagatgtcacaggtgacgatgacagtcccttacacatgtgtttttggagctcctcacaggtgacgatgacagtcccttacacaggtgacgatgacagtccctttctttttatttatctttttttttattattgtaagggcctcttagatttctcctataaaacgagagttagaaagatcaagaaaatggtgcacaaaaaaaaaaacgaaagatcaagaaaacaaaagagaataaaactgcaaagatacaaattatggagactgtctccgccgttaaccaaacactccccatctccggcggtgaaccggtgaagttcacgacatactctgccgcagttcacaaagtccttgtcatgatcaacgccggaattctagggttactccagcttgtcagccaacagtcctctgttttggaaacacataaagccgcattcctttgtttctgtgttttcattctattctacgccgttcttcgcgtccgtgaagccatggacgtgcgcctacaacccggtttagtcccaaggctcattggacatgggagccatctcttcggtggtctagccgctcttgtactcgtctccgtcgttagtaccgcattttctattgtcctttttcttctctggtttatctggctctccgccgtcgtctacttggagacaaacaaacccagtgcctgtccacctcagttaccaccagtttaaatggagactgtctccgccgttaaccaaacactccccatctccggcggtgaaccggtgaagttcacgacatactctgccgcagttcacaaagtccttgtcatgatcaacgccggaattctagggttactccagcttgtcagccaacagtcctctgttttggaaacacataaagccgcattcctttgtttctgtgttttcattctattctacgccgttcttcgcgtccgtgaagccatggacgtgcgcctacaacccggtttagtcccaaggctcattggacatgggagccatctcttcggtggtctagccgctcttgtactcgtctccgtcgttagtaccgcattttctattgtcctttttcttctctggtttatctggctctccgccgtcgtctacttggagacaaacaaacccagtgcctgtccacctcagttaccaccagtttaacatcttgtggttttatgaatggatgagtgtgagatgaaggttaatgtagaataacaccggtgacgttataaacaggccaatcgggtagagactgtatcttggtaactagatgatgtggaagaatattccaaatatatttagttgacgtgaaagaaacagcctataaatcgagaatgctttctatatatggcgatttaatatatatattttccttgggtgtttttcatactactagatttctgcagtatgctttggttatattattttactggtgaaatttacgtttattgaattgattggttcatacaaaaaccaatgttggcttctaatgggatttgtgatgactaaatgattcagttcacttttctttattgtttaacaaagatgcggacaatcaaaagaaaattaaacttaaaaaaaaacgcttcggtcggtttcatcgttaaactatatataaactctacaagtgttcatctaaaacattcaaaaaaataatgtaacaaaagtttaaaacacgtagtttcct

SEQ ID NO: 6 - DNA, 22 bp, synthetic construct
  source 1..22: mol_type = other DNA
aactctcccgctatgtatgtcg

SEQ ID NO: 7 - DNA, 20 bp, synthetic construct
  source 1..20: mol_type = other DNA
aaccctcgtagattggcaca

SEQ ID NO: 8 - DNA, 18 bp, synthetic construct
  source 1..18: mol_type = other DNA
caccgactacctgatgaa

SEQ ID NO: 9 - DNA, 17 bp, synthetic construct
  source 1..17: mol_type = other DNA
cagcttctccttgatgt

SEQ ID NO: 10 - DNA, 39 bp, synthetic construct
  source 1..39: mol_type = other DNA
acacgctgaagctagtcgacatggagactgtctccgccg

SEQ ID NO: 11 - DNA, 40 bp, synthetic construct
  source 1..40: mol_type = other DNA
tggtctttgtagtcttcgaattaaactggtggtaactgag

SEQ ID NO: 12 - DNA, 22 bp, synthetic construct
  source 1..22: mol_type = other DNA
gtgaaccggtgaagttcacgac

SEQ ID NO: 13 - DNA, 20 bp, synthetic construct
  source 1..20: mol_type = other DNA
gaggtggacaggcactgggt

SEQ ID NO: 14 - DNA, 40 bp, synthetic construct
  source 1..40: mol_type = other DNA
cgacggccagtgccaagcttagccacacaaactcccatct

SEQ ID NO: 15 - DNA, 43 bp, synthetic construct
  source 1..43: mol_type = other DNA
gcgcgcctcgagatcctctagaaatttgtatctttgcagtttt

SEQ ID NO: 16 - DNA, 19 bp, synthetic construct
  source 1..19: mol_type = other DNA
aagcctgaactcaccgcga

SEQ ID NO: 17 - DNA, 21 bp, synthetic construct
  source 1..21: mol_type = other DNA
gtttccactatcggcgagtac

SEQ ID NO: 18 - DNA, 46 bp, synthetic construct
  source 1..46: mol_type = other DNA
tcgaggtcgacggtatcgataagcttagccagacaaactcccatct

SEQ ID NO: 19 - DNA, 45 bp, synthetic construct
  source 1..45: mol_type = other DNA
ttcctcttcttctttggcatgaattcaatttgtatctttgcagtt

SEQ ID NO: 20 - DNA, 40 bp, synthetic construct
  source 1..40: mol_type = other DNA
ggccccccctcgaggtcgacagccacacaaactcccatct

SEQ ID NO: 21 - DNA, 40 bp, synthetic construct
  source 1..40: mol_type = other DNA
acggcggagacagtctccataatttgtatctttgcagttt

SEQ ID NO: 22 - DNA, 40 bp, synthetic construct
  source 1..40: mol_type = other DNA
ggccccccctcgaggtcgacatggagactgtctccgccgt

SEQ ID NO: 23 - DNA, 40 bp, synthetic construct
  source 1..40: mol_type = other DNA
cattaaagcaggactctagaaggaaactacgtgttttaaa